European Patent Application EP 4 796 628 A1, published August 26, 2026. Title: 耐酸马克斯克鲁维酵母菌株及其应用. Applicant: 中国石油化工股份有限公司. The sequence listing filed with the application follows.

SEQUENCE LISTING (5 sequences)

SEQ ID NO: 1 - protein, 1175 aa, synthetic construct
MSTQNDLAGLRDNSNLLGEKNKILVANRGEIPIRIFRTAHELSMKTVAIYSHEDRLSMHRLKADEAYVIGEPGKYTPVGAYLAIDEIIKIAQLHGVSFIHPGYGFLSENSEFAKKVADSGITWVGPPADVIDAVGDKVSARNLAERADVPVVPGTPGPIETVEEAVEFVEKYGYPVIIKAAFGGGGRGMRVVREGDDIADAFQRAKSEAVTAFGNGTCFVERFLDKPKHIEVQLLADHYGNVIHLFERDCSVQRRHQKVVEVAPAKTLPESVRNAILTDAVKLAKEAGYRNAGTAEFLVDNQNRHYFIEINPRIQVEHTITEEITGIDIVAAQIQIAAGASLEQLGLLQDRITTRGFAIQCRITTEDPSKNFQPDTGRIDVYRSAGGNGVRLDGGNAFAGSVISPHYDSMLVKCSCSGSTYEIVRRKMLRALIEFRIRGVKTNIPFLLTLLTHPVFKSGDYWTTFIDDTPQLFEMVSSQNRAQKLLHYLADLAVNGSSIKGQIGLPKLKTHPTIPHLHKADGSILDVSAKPPAGWRDVLLQHGPEEFAKQVRKFKGTLLMDTTWRDAHQSLLATRVRTYDLAAIAPTTAHALSGAFALECWGGATFDVSMRFLHEDPWERLRTLRKLVPNIPFQMLLRGANGVAYSSLPDNAIDHFVKQAKDNGVDIFRVFDALNDLEQLTVGVDAVKKAGGVVEATICYSGDMLAPGKKYNLDYYLDIVEQVVKRGTHILGIKDMAGTLKPSAAKLLIGSIRTKYPDLPIHVHTHDSAGTGVASMAACAFAGADVVDVATNSMSGMTSQPSVNALLAALDGEIDCNVNVSYISQLDAYWAEMRLLYSCFEADLKGPDPEVYVHEIPGGQLTNLLFQAQQLGLGEQWAETKRAYREANLLLGDVVKVTPTSKVVGDLAQFMVTNKLTSDDVKRLASSLDFPDSVMDFFEGLIGQPYGGFPEPLRSDVLKNKRRKLTKRPGLELAPFDLEGIKEDLTNRFGDIDDCDVASYNMYPKVYEDFRKIREKYGDLSVLPTKNFLSPPSIGEEIVVTIEQGKTLIIKPQAIGDLNKETGIREVYFELNGELRKVSVADRSQKVETISKPKADAHDPFQVGSPMAGVVVEVKVHKGSLISKGQPVAVLSAMKMEMVISSPSDGQVKEVLVKDGENVDASDLLVVLEEAPAKE

SEQ ID NO: 2 - protein, 335 aa, synthetic construct
MVSVAVLGSSGGIGQPLSLLLKLDPRVSSLRLYDLKMSHGIATDLSHMDSNSICEGFNTDEIALALKGAQIVVIPAGVPRKPGMSRDDLFKINAKIIKSLALQIAEHAPEARVLVISNPVNSLVPIVYETLKSVGKFEPGKVMGITTLDIIRSHTFLVDVLGRKAYSVEKLRSAVTVVGGHSGETIVPIFTDQKFYRRLRDRELYDAYVHRVQFGGDEVVKAKDGSGSATLSMAWAGYSFVKQLLNSLHLETGEDVHPIPTFVYLPGLPGGKELQQKLGTSVEFFAAPVKLSKGIVVEVEHDWVDKLNDAEKKLIAKCLPILDKNIKKGLAFSQQ

SEQ ID NO: 3 - protein, 469 aa, synthetic construct
MSVRMVSYRVETDAFGEIKVPADKYWGAQTQRSFQNFKIGGAREKMPEPIVKAFGVLKKSAAIVNENLGTLDPAVAEPIKKAADEVAQGKLMDHFPLVVFQTGSGTQSNMNANEVISNRAIELIGGELGSKQIHPNNHCNQAQSSNDTFPSVMHIAAVTEITRHLLPELVALKDALKKKSDEFQHIVKIGRTHLQDATPLTLGQEFSGYVQQVENGIIRVEQSLHHLKFLAQGGTAVGTGLNTKVGFAEKIAEQVSKETGIDFKTAPNKFEALAAHDAIVEASGALNTLAVSLFKIANDIRYLGSGPRCGYGELSLPENEPGSSIMPGKVNPTQNEALTQVCVQVMGNHAAITFAGASGQFELNVFKPVMISNLLSSIRLLGDASNSFRIHCVEGIQANEDRISKLLHESLMLVTALNPKIGYDAASKVAKNAHKKGITLKESALELGVLSSEEFDEWVIPEKMIGPKE

SEQ ID NO: 4 - protein, 1139 aa, synthetic construct
MVDGRSSASIVAVDPERAARERDAAARALLQDSPLHTTMQYATSGLELTVPYALKVVASADTFDRAKEVADEVLRCAWQLADTVLNSFNPNSEVSLVGRLPVGQKHQMSAPLKRVMACCQRVYNSSAGCFDPSTAPVAKALREIALGKERNNACLEALTQACTLPNSFVIDFEAGTISRKHEHASLDLGGVSKGYIVDYVIDNINAAGFQNVFFDWGGDCRASGMNARNTPWVVGITRPPSLDMLRNPPKEASYISVISLDNEALATSGDYENLIYTADDKPLTCTYDWKAKELMKPSQSNIAQVSVKCYSAMYADALATACFIKRDPAKVRQLLDGWRYVRDTVRDYRVYVRENERVAKMFEIATEDAEMRKRRISNTLPARVIVVGGGLAGLSAAIEAAGCGAQVVLMEKEAKLGGNSAKATSGINGWGTRAQAKASIVDGGKYFERDTYKSGIGGNTDPALVKTLSMKSADAIGWLTSLGVPLTVLSQLGGHSRKRTHRAPDKKDGTPLPIGFTIMKTLEDHVRGNLSGRITIMENCSVTSLLSETKERPDGTKQIRVTGVEFTQAGSGKTTILADAVILATGGFSNDKTADSLLREHAPHLVNFPTTNGPWATGDGVKLAQRLGAQLVDMDKVQLHPTGLINPKDPANPTKFLGPEALRGSGGVLLNKQGKRFVNELDLRSVVSKAIMEQGAEYPGSGGSMFAYCVLNAAAQKLFGVSSHEFYWKKMGLFVKADTMRDLAALIGCPVESVQQTLEEYERLSTSQRSCPITRKSVYPCVLGTKGPYYVAFVTPSIHYTMGGCLISPSAEIQMKNTSSRAPLSHSNPILGLFGAGEVTGGVHGGNRLGGNSLLECVVFGRIAGDRASTILQRKSSALSFKVWTTVVLREVREGGVYGAGSRVLRFNLPGALQRSGLSLGQFIAIRGDWDGQQLIGYYSPITLPDDLGMIDILARSDKGTLREWISALEPGDAVEMKACGGLVIERRLSDKHFVFMGHIINKLCLIAGGTGVAPMLQIIKAAFMKPFIDTLESVHLIYAAEDVTELTYREVLEERRRESRGKFKKTFVLNRPPPLWTDGVGFIDRGILTNHVQPPSDNLLVAICGPPVMQRIVKATLKTLGYNMNLVRTVDETEPSGS

SEQ ID NO: 5 - DNA, 3420 bp, synthetic construct
  source 1..3420: mol_type = other DNA
atggtcgatggtagatcttctgcttctatcgttgctgttgacccagaaagagctgctagagaaagagacgctgctgctagagctttgttgcaagactccccattgcacaccaccatgcaatacgctacttccggtttggaattgaccgttccatacgctttgaaggttgttgcttccgctgacaccttcgacagagctaaggaagttgctgacgaagttttgagatgtgcttggcaattggctgacactgttttgaactctttcaacccaaactctgaagtttctttggttggtagattgccagttggtcaaaagcaccaaatgtctgctccattgaagagagttatggcttgttgtcaaagagtttacaactcttctgctggttgtttcgacccatctactgctccagttgctaaggctttgagagaaatcgctttgggtaaggaaagaaacaacgcttgtttggaagctctaactcaagcctgtaccttgccaaactctttcgttattgacttcgaagctggtactatctctagaaagcacgaacacgcttctttggacttgggtggtgtctctaagggttacattgtcgattacgttattgacaacattaacgctgctggtttccaaaacgttttcttcgactggggtggtgactgtagagcttctggtatgaacgctagaaacaccccatgggttgttggtattaccagaccaccatctttggacatgttgagaaacccaccaaaggaagctagttacatctctgttatttctttggataacgaagctctagctacctctggtgactacgaaaacttgatctacaccgctgacgacaagccattgacctgtacctacgactggaaggctaaggaattgatgaagccatcccaatctaacatcgctcaagtttctgttaagtgttactctgctatgtacgctgacgctttggctaccgcttgtttcatcaagagagatccagctaaggttagacaattgttggacggttggagatacgttagagacaccgttagagactacagagtttacgttagagaaaacgaaagagttgctaagatgttcgaaatcgctaccgaagacgctgaaatgagaaagagaagaatctctaacaccttgccagctagagttatcgttgttggtggtggtttggctggtttgtctgctgctattgaagctgctggttgtggtgctcaagttgttttgatggaaaaggaagctaagttgggtggtaactctgctaaggctacctctggtattaacggttggggtactagagctcaagctaaggcttctattgttgacggtggtaagtacttcgaaagagacacctacaagtccggtattggtggtaacactgacccagctttggttaagaccttgtctatgaagtccgctgacgctatcggttggttgacctctttgggtgtcccattgaccgttttgtcccaattgggtggtcactctagaaagagaacccatagagctccagacaagaaggacggtactccattgccaattggtttcactatcatgaagactttggaagaccacgtcagaggtaacttgtctggtagaatcaccatcatggaaaactgttccgttacctctttgttgtctgaaaccaaggaaagaccagacggtactaagcaaatcagagttaccggtgttgaatttactcaagctggttctggtaagaccaccatcttggctgacgctgttatcttggctaccggtggtttctctaacgacaagactgctgactctttgttgagagaacacgctccacacttggttaacttcccaaccactaacggtccatgggctactggtgatggtgttaagttggctcaaagattgggtgctcaattggttgacatggacaaggttcaattgcacccaaccggtttgatcaacccaaaggacccagctaacccaaccaagttcttgggtccagaagctctaagaggttccggtggtgttttgttgaacaagcaaggtaagagattcgttaacgaattggatttgagatccgttgtttctaaggctatcatggaacaaggtgctgaatacccaggttctggtggttctatgttcgcttactgtgtcttgaacgctgctgctcaaaagttgttcggtgtttcttctcacgaattttactggaagaagatgggtttgttcgttaaggctgatactatgagagatttggctgctttgatcggttgtccagttgaatctgttcaacaaactttggaagaatacgaaagattgtctacctctcaaagatcttgtccaattaccagaaagtctgtttacccatgtgttttgggtactaagggtccatactacgttgctttcgttaccccatctattcactacaccatgggtggttgtttgatctctccatctgctgaaatccaaatgaagaacacctcttctagagctccattgtctcactctaacccaattttgggtttgttcggtgctggtgaagttaccggtggtgttcacggtggtaacagattgggtggtaactccttgttggaatgtgttgttttcggtagaatcgctggtgacagagcttctactattttgcaaagaaagtcttctgctttgtctttcaaggtttggactactgttgttttgagagaagttagagaaggtggtgtttacggtgctggttctagagttttgagattcaacttgccaggtgctttgcaaagatctggtttgtctttgggtcaattcatcgctattagaggtgactgggatggtcaacaattgatcggttactactctccaatcaccttgccagacgacttgggtatgatcgacattttggctagatctgataagggtactttgagagaatggatttctgctttggaaccaggtgacgctgttgaaatgaaggcttgtggtggtttggttattgaaagaagattgtccgacaagcatttcgttttcatgggtcatatcatcaacaagttgtgtttgatcgctggtggtactggtgttgctccaatgttgcaaattattaaggctgctttcatgaagccattcatcgacaccttggaatctgttcacttgatctacgctgctgaagacgttaccgaattgacttacagagaagttttggaagaaagaagaagagaatctagaggtaagttcaagaagaccttcgttttgaacagaccaccaccattgtggaccgatggtgttggtttcatcgacagaggtatcttgaccaaccacgttcaaccaccatccgacaacttgttggttgctatctgtggtccaccagttatgcaaagaatcgttaaggctaccttgaagaccttgggttacaacatgaacttggttagaaccgttgacgaaaccgaaccatctggttcctaa